European Patent Application EP 4 790 147 A1, published August 12, 2026. Title: 新型DNA甲基化标志物TAGMe-6及其作为肿瘤诊断靶点的用途. Applicant: 上海奕谱生物科技有限公司. Application CN. The sequence listing filed with the application follows.

SEQUENCE LISTING (30 sequences)

SEQ ID NO: 1 - DNA, 1731 bp, Homo sapiens
  source 1..1731: mol_type = genomic DNA
ggctcctgcagctcccgccgaagactcaaagccagagtggacataaacgccgtgggcaggaccccggtgaggcctcggtgcccttcttgggggttctcagcgttggcccagaagcctcagcccgggtctaagaacttgggactctcctcgactttggcgatcggccgggtcatccggctcagggcctcagcggcagcgggcaaaactctagtaggagtctcttgccgagggcgtgtttcgacgtcagagccaaactcgggacagactagccaagcgcggacggcgcgagagtggctggcagcgccagcacgcagcctgggttcagagcaaggctgggcgctctcagcaaagggcggcctggggctgcgcgggcggcggactgcaggcgggagaagagcgaggtgcgccaggctctggggcgcgcaactgcccagcctcgtgaaagatcgcgccgcagatggggcgcagctgcgcgctcactcgtgtggactggaaacgctccgagccggttattttaaaaaccgggaaataaggcgggttccctcttcgcccgccacttcccaccaagtaggctgtgcggccctgggggctgactgtcctcaagcagccaggctccaccgcgcgccgcgctgcgccgaggtccgctctgccgcagggacgctggcagcccgttgaacaccggcaagagcgccagaggctagcggccgccaggatctctaccaggctctgctcgcacccgcctgcctccctttcgtttggcctgtcctccgttcaactgaaatcgttaattttcttacccccttgttctcattttgatatattctacgctttaaacatgctccgttttcttttgtttagtctgctccctccctctttgtcctttcccccttctctagttatccgtttcgttcgatcttgctcctgctttttttattcgttcgttcctcatttattcattttagttcatcccagctcgccgactgccatttaccctctcgttctcgccgcgctctccgttgttttgttcaatttcccttccccttttcttggttgtcgctcgctttctttggttttctttctcggtatttcgttgtcaaggccacccttgccgtcggatcccggggtgctgggtttctcccggccgctcgttccgcaccagcgctctctgcagttcgcgcggcaccggtgtggtccgggggcccgagctgtcggtgccggatgcggcgcgcctagcagggacgcgggcctgggggggtggctcctgcccgacgcggagcgctgagccaggccgggtacctgtctctggcggtgctcaccgcactgcgcggcctctgccgtctggctgggatcagaggagccaggccaactgcttctcattaagtcccaactgtggtttttatcaggaaagcctctttcaaagggcacagacacgaagctccgcggactcgttcatttcctccgttgacccacacacacctccccgccctcccctacacattcccaccgccccggctgggcgaaagccggagatgcccggccactccgtggaggcccgcgaggcgccagccgggcggcggcagggggttgaggcggatcttggaggatccagttctgggcctaggctgcgggatatggcagcgcagataaggtgggtgcagtgcggaagccgagacgccttacaggtcatagggtgcggcggacggccgcagagctgccgatcagcctgccagg

SEQ ID NO: 2 - DNA, 1731 bp, synthetic construct
  source 1..1731: mol_type = other DNA
ggtttttgtagttttygtygaagatttaaagttagagtggatataaaygtygtgggtaggatttyggtgaggtttyggtgttttttttgggggtttttagygttggtttagaagttttagttygggtttaagaatttgggatttttttygattttggygatyggtygggttattyggtttagggttttagyggtagygggtaaaattttagtaggagttttttgtygagggygtgtttygaygttagagttaaattygggatagattagttaagygyggayggygygagagtggttggtagygttagtaygtagtttgggtttagagtaaggttgggygtttttagtaaagggyggtttggggttgygygggyggyggattgtaggygggagaagagygaggtgygttaggttttggggygygtaattgtttagtttygtgaaagatygygtygtagatggggygtagttgygygtttattygtgtggattggaaaygtttygagtyggttattttaaaaatygggaaataaggygggtttttttttygttygttattttttattaagtaggttgtgyggttttgggggttgattgtttttaagtagttaggttttatygygygtygygttgygtygaggttygttttgtygtagggaygttggtagttygttgaatatyggtaagagygttagaggttagyggtygttaggatttttattaggttttgttygtattygtttgtttttttttygtttggtttgtttttygtttaattgaaatygttaatttttttatttttttgtttttattttgatatattttaygttttaaatatgtttygtttttttttgtttagtttgttttttttttttttgtttttttttttttttttagttattygtttygttygattttgtttttgttttttttattygttygttttttatttatttattttagtttattttagttygtygattgttatttattttttygttttygtygygtttttygttgttttgtttaatttttttttttttttttttggttgtygttygttttttttggttttttttttyggtatttygttgttaaggttatttttgtygtyggatttyggggtgttgggtttttttyggtygttygtttygtattagygttttttgtagttygygyggtatyggtgtggttygggggttygagttgtyggtgtyggatgyggygygtttagtagggaygygggtttgggggggtggtttttgttygaygyggagygttgagttaggtygggtatttgtttttggyggtgtttatygtattgygyggtttttgtygtttggttgggattagaggagttaggttaattgttttttattaagttttaattgtggtttttattaggaaagttttttttaaagggtatagataygaagtttygyggattygtttatttttttygttgatttatatatattttttygtttttttttatatatttttatygtttyggttgggygaaagtyggagatgttyggttatttygtggaggttygygaggygttagtygggyggyggtagggggttgaggyggattttggaggatttagttttgggtttaggttgygggatatggtagygtagataaggtgggtgtagtgyggaagtygagaygttttataggttatagggtgyggyggayggtygtagagttgtygattagtttgttagg

SEQ ID NO: 3 - DNA, 58 bp, synthetic construct
  source 1..58: mol_type = other DNA
tacacgacgctcttccgatctcgtgatygttgattgtttttaagtagttaggttttat

SEQ ID NO: 4 - DNA, 55 bp, synthetic construct
  source 1..55: mol_type = other DNA
gacgtgtgctcttccgatcttagcttraacaaaacctaataaaaatcctaacrac

SEQ ID NO: 5 - DNA, 58 bp, synthetic construct
  source 1..58: mol_type = other DNA
aatgatacggcgaccaccgagatctacactctttccctacacgacgctcttccgatct

SEQ ID NO: 6 - DNA, 64 bp, synthetic construct
  source 1..64: mol_type = other DNA
caagcagaagacggcatacgagatcgtgatgtgactggagttcagacgtgtgctcttccgatct

SEQ ID NO: 7 - DNA, 28 bp, synthetic construct
  source 1..28: mol_type = other DNA
tacacgacgctcttccgatctcgtgaty

SEQ ID NO: 8 - DNA, 28 bp, synthetic construct
  source 1..28: mol_type = other DNA
tacacgacgctcttccgatctacatcgy

SEQ ID NO: 9 - DNA, 28 bp, synthetic construct
  source 1..28: mol_type = other DNA
tacacgacgctcttccgatctgcctaay

SEQ ID NO: 10 - DNA, 28 bp, synthetic construct
  source 1..28: mol_type = other DNA
tacacgacgctcttccgatcttggtcay

SEQ ID NO: 11 - DNA, 28 bp, synthetic construct
  source 1..28: mol_type = other DNA
tacacgacgctcttccgatctcactgty

SEQ ID NO: 12 - DNA, 28 bp, synthetic construct
  source 1..28: mol_type = other DNA
tacacgacgctcttccgatctattggcy

SEQ ID NO: 13 - DNA, 28 bp, synthetic construct
  source 1..28: mol_type = other DNA
tacacgacgctcttccgatctgatctgy

SEQ ID NO: 14 - DNA, 28 bp, synthetic construct
  source 1..28: mol_type = other DNA
tacacgacgctcttccgatcttcaagty

SEQ ID NO: 15 - DNA, 28 bp, synthetic construct
  source 1..28: mol_type = other DNA
tacacgacgctcttccgatctctgatcy

SEQ ID NO: 16 - DNA, 28 bp, synthetic construct
  source 1..28: mol_type = other DNA
tacacgacgctcttccgatctaagctay

SEQ ID NO: 17 - DNA, 27 bp, synthetic construct
  source 1..27: mol_type = other DNA
gacgtgtgctcttccgatcttagcttr

SEQ ID NO: 18 - DNA, 27 bp, synthetic construct
  source 1..27: mol_type = other DNA
gacgtgtgctcttccgatctggctacr

SEQ ID NO: 19 - DNA, 27 bp, synthetic construct
  source 1..27: mol_type = other DNA
gacgtgtgctcttccgatctcttgtar

SEQ ID NO: 20 - DNA, 27 bp, synthetic construct
  source 1..27: mol_type = other DNA
gacgtgtgctcttccgatctagtcaar

SEQ ID NO: 21 - DNA, 27 bp, synthetic construct
  source 1..27: mol_type = other DNA
gacgtgtgctcttccgatctagttccr

SEQ ID NO: 22 - DNA, 27 bp, synthetic construct
  source 1..27: mol_type = other DNA
gacgtgtgctcttccgatctccgaccr

SEQ ID NO: 23 - DNA, 27 bp, synthetic construct
  source 1..27: mol_type = other DNA
gacgtgtgctcttccgatctggacggr

SEQ ID NO: 24 - DNA, 27 bp, synthetic construct
  source 1..27: mol_type = other DNA
gacgtgtgctcttccgatctctctacr

SEQ ID NO: 25 - DNA, 27 bp, synthetic construct
  source 1..27: mol_type = other DNA
gacgtgtgctcttccgatctgcggacr

SEQ ID NO: 26 - DNA, 27 bp, synthetic construct
  source 1..27: mol_type = other DNA
gacgtgtgctcttccgatcttgtgatr

SEQ ID NO: 27 - DNA, 25 bp, synthetic construct
  source 1..25: mol_type = other DNA
ggtttttgtagttttygtygaagat

SEQ ID NO: 28 - DNA, 25 bp, synthetic construct
  source 1..25: mol_type = other DNA
acctaactacttaaaaacaatcaac

SEQ ID NO: 29 - DNA, 25 bp, synthetic construct
  source 1..25: mol_type = other DNA
gttaggatttttattaggttttgtt

SEQ ID NO: 30 - DNA, 25 bp, synthetic construct
  source 1..25: mol_type = other DNA
cctaacaaactaatcracaactcta